European Patent Specification EP 3 733 699 B1, published June 24, 2026. Title: A FULLY NATIVE HUMAN NEUTRALIZING MONOCLONAL ANTIBODY AGAINST TETANUS TOXIN AND ITS APPLICATIONS. Applicant: ZHUHAI TRINOMAB BIOTECHNOLOGY CO., LTD. The sequence listing filed with the application follows.

SEQUENCE LISTING (34 sequences)

SEQ ID NO: 1 - protein, 8 aa, Artificial Sequence
  antibody sequence
GGSISSYY

SEQ ID NO: 2 - protein, 7 aa, Artificial Sequence
  antibody sequence
VHYSGST

SEQ ID NO: 3 - protein, 12 aa, Artificial Sequence
  antibody sequence
ARDKYQTDVSDI

SEQ ID NO: 4 - protein, 7 aa, Artificial Sequence
  antibody sequence
QSITSSF

SEQ ID NO: 5 - protein, 3 aa, Artificial Sequence
  antibody sequence
GAS

SEQ ID NO: 6 - protein, 8 aa, Artificial Sequence
  antibody sequence
QQYDTSRT

SEQ ID NO: 7 - protein, 118 aa, Artificial Sequence
  antibody sequence
QVQLQESGPGLVKPSETLSLRCTVSGGSISSYYWSWFRQPPGKGLEWIGYVHYSGSTNYNPSLKSRFTLSVDTSKSQFSLRLRSVTAADTAIYYCARDKYQTDVSDIWGQGTVVTVSS

SEQ ID NO: 8 - protein, 107 aa, Artificial Sequence
  antibody sequence
DIQMTQSPGTLSLSPGERATLSCRASQSITSSFLAWYQQKPGQAPRLLIYGASSRATGIPDRFSGSGSGTDFILTISRLEPEDFAVYYCQQYDTSRTFGQGTTVEIK

SEQ ID NO: 9 - protein, 8 aa, Artificial Sequence
  antibody sequence
GYTFTNYW

SEQ ID NO: 10 - protein, 8 aa, Artificial Sequence
  antibody sequence
VYPGDSDT

SEQ ID NO: 11 - protein, 18 aa, Artificial Sequence
  antibody sequence
ATQQSNPYDSGSYWYFDS

SEQ ID NO: 12 - protein, 89 aa, Artificial Sequence
  antibody sequence
GYTFTNYWIGWVRQMPGKGLEWMGIVYPGDSDTRYSPSFQGQITISADKSISTAYLQWNNLKASDTGMYYCATQQSNPYDSGSYWYFDS

SEQ ID NO: 13 - protein, 6 aa, Artificial Sequence
  antibody sequence
QGIRNF

SEQ ID NO: 14 - protein, 3 aa, Artificial Sequence
  antibody sequence
AAS

SEQ ID NO: 15 - protein, 9 aa, Artificial Sequence
  antibody sequence
QKYFSAPPD

SEQ ID NO: 16 - protein, 71 aa, Artificial Sequence
  antibody sequence
QGIRNFLAWYQQKPGKVPKLLIYAASTLQSGVPSRFSGSGSGTDFTLTISSLQPEDVATYYCQKYFSAPPD

SEQ ID NO: 17 - protein, 125 aa, Artificial Sequence
  antibody sequence
EVQLVQSGAEVKKPGESLRISCQGSGYTFTNYWIGWVRQMPGKGLEWMGIVYPGDSDTRYSPSFQGQITISADKSISTAYLQWNNLKASDTGMYYCATQQSNPYDSGSYWYFDSWGQGTLVTVSS

SEQ ID NO: 18 - protein, 107 aa, Artificial Sequence
  antibody sequence
DIVMTQSPPSLSASIGDRVTITCRASQGIRNFLAWYQQKPGKVPKLLIYAASTLQSGVPSRFSGSGSGTDFTLTISSLQPEDVATYYCQKYFSAPPDFGQGTRLEIK

SEQ ID NO: 19 - protein, 8 aa, Artificial Sequence
  antibody sequence
GGPFTGSY

SEQ ID NO: 20 - protein, 7 aa, Artificial Sequence
  antibody sequence
VSQSGST

SEQ ID NO: 21 - protein, 12 aa, Artificial Sequence
ARLTKHYINSAY

SEQ ID NO: 22 - protein, 118 aa, Artificial Sequence
  antibody sequence
QVQLQESGAGLVKPSETLSLTCGVAGGPFTGSYLSWIRQPPGKGLEWIGEVSQSGSTSYNPSLKSRVTISVDTSKSQFSLKLSSVTAADTAVYYCARLTKHYINSAYWGQGTLVTVSS

SEQ ID NO: 23 - protein, 6 aa, Artificial Sequence
  antibody sequence
QIIGSW

SEQ ID NO: 24 - protein, 3 aa, Artificial Sequence
KAS

SEQ ID NO: 25 - protein, 9 aa, Artificial Sequence
  antibody sequence
QQYNSYPYT

SEQ ID NO: 26 - protein, 107 aa, Artificial Sequence
  antibody sequence
DIQMTQSPSILSASVGDRVTITCRASQIIGSWLAWYQQKPGKAPTLVIYKASRLDSGVPSRFSGTESGTEFTLTISSLQPDDFATYYCQQYNSYPYTFGQGTKLEIK

SEQ ID NO: 27 - protein, 8 aa, Artificial Sequence
  antibody sequence
GFGIGIYT

SEQ ID NO: 28 - protein, 8 aa, Artificial Sequence
  antibody sequence
ISGTSQYI

SEQ ID NO: 29 - protein, 8 aa, Artificial Sequence
  antibody sequence
VSGSSLDY

SEQ ID NO: 30 - protein, 6 aa, Artificial Sequence
  antibody sequence
QNIGTN

SEQ ID NO: 31 - protein, 3 aa, Artificial Sequence
  antibody sequence
GAS

SEQ ID NO: 32 - protein, 9 aa, Artificial Sequence
  antibody sequence
YQNYNSPKT

SEQ ID NO: 33 - protein, 115 aa, Artificial Sequence
  antibody sequence
EVQLVESGGGRVKPGGSLRLSCSVSGFGIGIYTMNWVRQAPGKGLEWVSSISGTSQYIYYANSVRGRFTISRDNAENSLYLQLNNLRAEDTALYYCVSGSSLDYWGQGTLVTISS

SEQ ID NO: 34 - protein, 107 aa, Artificial Sequence
  antibody sequence
DIQLTQSPSSLSASVGGRVTITCRASQNIGTNLNWFQQKPGTAPNLLIYGASTLQSGVPSRFSGSGSGTTFTLTIDSLQPEDFATYYCYQNYNSPKTFGQGTKVDLK